European Patent Application EP 4 317 458 A1, published February 7, 2024. Title: Follicular Thyroid Cancer-Specific Marker. Applicant: Nippon Medical School Foundation University Public Corporation Osaka. The sequence listing filed with the application follows.

SEQUENCE LISTING (6 sequences)

SEQ ID NO: 1 - DNA, 72 bp, Homo sapiens
tttgtacttcaggtgcacagaattggattaataataatccgtggcttataacatactctcagcattggtaat

SEQ ID NO: 2 - DNA, 20 bp, Artificial
  Forward Primer
gtacttcaggtgcacagaat

SEQ ID NO: 3 - DNA, 20 bp, Artificial
  Reverse Primer
atactctcagcattggtaat

SEQ ID NO: 4 - DNA, 20 bp, Artificial
  Forward Primer
aggagcatcgctaggtgttg

SEQ ID NO: 5 - DNA, 22 bp, Artificial
  Reverse Primer
atctcttactcatcctgcagcc

SEQ ID NO: 6 - DNA, 15 bp, Artificial
  Probe
cgccaccgggaagcg